European Patent Application EP 4 317 407 A1, published February 7, 2024. Title: CELL CULTURE SUBSTRATE, METHOD FOR PRODUCING THE SAME, METHOD FOR INDUCING DIFFERENTIATION OF PLURIPOTENT STEM CELL AND KIT FOR CELL CULTURE. Applicant: TOSOH CORPORATION. The sequence listing filed with the application follows.

SEQUENCE LISTING (4 sequences)

SEQ ID NO: 1 - DNA, 41 bp, Homo sapiens
acatcgctcagacaccatgtgtagttgaggtcaatgaaggg

SEQ ID NO: 2 - DNA, 41 bp, Homo sapiens
gctggagaaggagtttcactacctttgctctgcggttctga

SEQ ID NO: 3 - DNA, 42 bp, Homo sapiens
ttgccacaattccctgagatgatgttgagagagcctttgact

SEQ ID NO: 4 - DNA, 41 bp, Homo sapiens
ggaatgtttcaggctcaagatgtcaagcaggtgttcacagg